European Patent Specification EP 2 590 673 B1, published May 21, 2025. Title: Designer Peptide-Based PCV2 Vaccine. Applicant: United Biomedical Inc Wang, Chang Yi Wen-Jiun, Peng. Application TBD. The sequence listing filed with the application follows.

SEQUENCE LISTING (20 sequences)

SEQ ID NO: 1 - protein, 154 aa, Porcine circovirus - type 2 strain Cyc08 from Taiwan
TRLSRTFGYTVKATTVRTPSWAVDMMRFNISDFVPPGGGTNKISIPFEYYRIRKVKVEFWPCSPITQGDRGVGSTAVILDDNFVTKATALTYDPYVNYSSRHTIPQPFSYHSRYFTPKPVLDSTIDYFQPNNKRNQLWLRLQTSANVDHVGLGT

SEQ ID NO: 2 - protein, 19 aa, Measles virus - Modified T helper site
  MISC_FEATURE (4)..(4): S or T
  MISC_FEATURE (7)..(7): K or R
  MISC_FEATURE (8)..(8): G or T
  MISC_FEATURE (12)..(12): H or T
  MISC_FEATURE (13)..(13): K or R
ISIXEIXXVIVXXIETILF

SEQ ID NO: 3 - protein, 20 aa, Porcine circovirus
CHIEKAKGTDQQNKEYCSKE

SEQ ID NO: 4 - protein, 20 aa, Porcine circovirus
KWWDGYHGEEVVVIDDFYGW

SEQ ID NO: 5 - protein, 20 aa, Porcine circovirus
PRWPHNDVYIGLPITLLHFP

SEQ ID NO: 6 - protein, 177 aa, Artificial Sequence
  B cell epitope cluster peptide derived from PCV2 ORF2 capsid protein (Cap1 peptide) linked through spacer to artificial combinatorial Th peptide (UBITh3)
  MISC_FEATURE (4)..(4): S or T
  MISC_FEATURE (7)..(7): K or R
  MISC_FEATURE (8)..(8): G or T
  MISC_FEATURE (12)..(12): H or T
  MISC_FEATURE (13)..(13): K or R
  MOD_RES (23)..(23): AMIDATION
  MISC_FEATURE (23)..(23): (epsilonN)Lys
ISIXEIXXVIVXXIETILFKKKXTRLSRTFGYTVKATTVRTPSWAVDMMRFNISDFVPPGGGTNKISIPFEYYRIRKVKVEFWPCSPITQGDRGVGSTAVILDDNFVTKATALTYDPYVNYSSRHTIPQPFSYHSRYFTPKPVLDSTIDYFQPNNKRNQLWLRLQTSANVDHVGLGT

SEQ ID NO: 7 - protein, 4 aa, artificial
  artificial spacer sequence
  MOD_RES (4)..(4): AMIDATION
  MISC_FEATURE (4)..(4): (epsilonN)Lys
KKKX

SEQ ID NO: 8 - DNA, 24 bp, Artificial Sequence
  CpG oligo nucleotide
tcgtcgttttgtcgttttgtcgtt

SEQ ID NO: 9 - protein, 154 aa, Porcine circovirus - US
TRLSRTFGYTIKRTTVRTPSWAVDMMRFNINDFLPPGGGSNPRSVPFEYYRIRKVKVEFWPCSPITQGDRGVGSSAVILDDNFVTKATALTYDPYVNYSSRHTITQPFSYHSRYFTPKPVLDSTIDYFQPNNKRNQLWLRLQTAGNVDHVGLGT

SEQ ID NO: 10 - protein, 154 aa, Porcine circovirus - DK
TRLSRTFGYTIKRTTVKTPSWAVDMMRFNINDFLPPGGGSNPRSVPFEYYRIRKVKVEFWPCSPITQGDRGVGSSAVILDDNFVTKATALTYDPYVNYSSRHTITQPFSYHSRYFTPKPVLDSTIDYFQPNNKRNQLWLRLQTAGNVDHVGLGT

SEQ ID NO: 11 - protein, 154 aa, Porcine circovirus - DE
TRLSRTFGYTIKRTTVKTPSWAVDMMRFNINDFLPPGGGSNPRSVPFEYYRIRKVKVEFWPCSPITQGDRGVGSSAVILDDNFVTKATALTYDPYVNYSSRHTITQPFSYHSRYFTPKPVLDSTIDYFQPNNKRNQLWMRLQTSRNVDHVGLGT

SEQ ID NO: 12 - protein, 150 aa, Porcine circovirus - ES
RTFGYTVKRTPVRTPSWAVDMMRFNINDFLPPGGGSNHRSVPFEYYRIRKVKVEFWPCSPITQGDRGVGSSAVILDDNFVTKATALTYDPYVNYSSRHTITQPFSYHSRYFTPKPVLDSTIDYFQPNNKRNQLWLRLQTAGNVDHVGLGT

SEQ ID NO: 13 - protein, 154 aa, Porcine circovirus - CN
TRLSRTIGYTVKKTTVRTPSWNVDMMRFNINDFLPPGGGSNPLTVPFEYYRIRKVKVEFWPCSPITQGDRGVGSTAVILDDNFVTKANALTYDPYVNYSSRHTITQPFSYHSRYFTPKPVLDRTIDYFQPNNKRNQLWLRLQTTGNVDHVGLGT

SEQ ID NO: 14 - protein, 154 aa, Porcine circovirus - CN
TRLSRTIGYTVKKTTVRTPSWNVDMMRFNINDFLPPGGGSNPLTMPFEYYRIRKVKVEFWPCSPITQGDRGVGSTAVILDDNFVTKANALTYDPYVNYSSRHTITQPFSYHSRYFTPKPVLDRTIDYFQPNNKRNQLWLRLQTTGNVDHVGLGT

SEQ ID NO: 15 - protein, 154 aa, Porcine circovirus - CN
ARLSRTFGYTVKRTTVTTPSWAVDMMRFKLDDFVPPGGGTNKISIPFEYYRIRKVKVEFWPCSPITQGDRGVGSTAVILDDNFVPKANALTYDPYVNYSFRHTIPQPFSYHSRYFTPKPVLDSTIDYFQPNNKRNQLWMRIQTSRNVDHVGLGT

SEQ ID NO: 16 - protein, 154 aa, Porcine circovirus - BR
TRLSRTFGYTVKRTTVTTPSWAVDMMRFKLDDFVPPGGGTNKISIPFEYYRIRKVKVEFWPCSPITQGDRGVGSTAVILDDNFVPKANALTYDPYVNYSSRHTIPQPFSYHSRYFTPKPVLDSTIDYFQPNNKKNQLWLRLQTSRNVDHVGLGT

SEQ ID NO: 17 - protein, 154 aa, Porcine circovirus - US
ARLSRTFGYTVKATTVSTPSWAVDMMRFNLDDFVPPGGGTNKISIPFEYYRIRKVKVEFWPCSPITQGDRGVGSSAIILDDNFVIKATAQTYDPYVNYSSRHTIPQPFSYHSRYFTPKPVLDSTIDYFQPNNKRNQLWMRLQTSRNVDHVGLGT

SEQ ID NO: 18 - protein, 154 aa, Porcine circovirus - CA
TRLSRTFGYTVKATTVRTPSWAVDMMRFNIDDFVPPGGGTNKISIPFEYYRIRKVKVEFWPCSPITQGDRGVGSTAVILDDNFVTKATALTYDPYVNYSSRHTIPQPFSYHSRYFTPKPVLDSTIDYFQPNNKRNQLWMRLQTSRNVDHVGLGT

SEQ ID NO: 19 - protein, 154 aa, Porcine circovirus - TW
TRLSRTFGYTVKATTVRTPSWAVDMMRFNINDFVPPGGGTNKISIPFEYYRIRKVKVEFWPCSPITQGDRGVGSTAVILDDNFVTKATALTYDPYVNYSSRHTIPQPFSYHSRYFTPKPVLDSTIDYFQPNNKRNQLWLRLQTSANVDHVGLGT

SEQ ID NO: 20 - protein, 154 aa, Artificial Sequence
  Porcine circovirus - consensus sequence
TRLSRTFGYTVKRTPVRTPSWAVDMMRFNINDFLPPGGGSNHRSIPFEYYRIRKVKVEFWPCSPITQGDRGVGSTAVILDDNFVTKATALTYDPYVNYSSRHTITQPFSYHSRYFTPKPVLDSTIDYFQPNNKRNQLWLRLQTSANVDHVGLGT